European Patent Application EP 4 410 813 A1, published August 7, 2024. Title: Peptide having hair loss preventing activity or hair growth promoting activity and use thereof. Applicant: CAREGENE CO., LTD. The sequence listing filed with the application follows.

SEQUENCE LISTING (21 sequences)

SEQ ID NO: 1 - protein, 6 aa, synthetic construct
HLPKPI

SEQ ID NO: 2 - DNA, 20 bp, synthetic construct
  source 1..20: mol_type = other DNA
ccagctattgtaacacctca

SEQ ID NO: 3 - DNA, 20 bp, synthetic construct
  source 1..20: mol_type = other DNA
ttcagatgtaggcagctgtc

SEQ ID NO: 4 - DNA, 25 bp, synthetic construct
  source 1..25: mol_type = other DNA
accagcagcgactctgaggaggaac

SEQ ID NO: 5 - DNA, 26 bp, synthetic construct
  source 1..26: mol_type = other DNA
tgaccctcttggcagcaggatagtcc

SEQ ID NO: 6 - DNA, 28 bp, synthetic construct
  source 1..28: mol_type = other DNA
accttcgttgccctctgtgccacagatg

SEQ ID NO: 7 - DNA, 21 bp, synthetic construct
  source 1..21: mol_type = other DNA
aggcccggaggcagtccgggt

SEQ ID NO: 8 - DNA, 20 bp, synthetic construct
  source 1..20: mol_type = other DNA
ggagccaaaagggtcatcat

SEQ ID NO: 9 - DNA, 20 bp, synthetic construct
  source 1..20: mol_type = other DNA
gtgatggcatggactgtggt

SEQ ID NO: 10 - DNA, 20 bp, synthetic construct
  source 1..20: mol_type = other DNA
gatcatcgagctgagacgca

SEQ ID NO: 11 - DNA, 20 bp, synthetic construct
  source 1..20: mol_type = other DNA
ctggccccagggtatctagt

SEQ ID NO: 12 - DNA, 20 bp, synthetic construct
  source 1..20: mol_type = other DNA
ccctcaaggatgccaggaac

SEQ ID NO: 13 - DNA, 19 bp, synthetic construct
  source 1..19: mol_type = other DNA
cactgctacctccggcaag

SEQ ID NO: 14 - DNA, 20 bp, synthetic construct
  source 1..20: mol_type = other DNA
ccaaatccgcaccaaggtca

SEQ ID NO: 15 - DNA, 21 bp, synthetic construct
  source 1..21: mol_type = other DNA
gtattgattgccaggaggggg

SEQ ID NO: 16 - DNA, 20 bp, synthetic construct
  source 1..20: mol_type = other DNA
cgcggcgtatccgtgtcctc

SEQ ID NO: 17 - DNA, 24 bp, synthetic construct
  source 1..24: mol_type = other DNA
agcctgttccgtctcaaacttggt

SEQ ID NO: 18 - DNA, 20 bp, synthetic construct
  source 1..20: mol_type = other DNA
cggtcaagtcggaaaattca

SEQ ID NO: 19 - DNA, 20 bp, synthetic construct
  source 1..20: mol_type = other DNA
gaggagctgggatgtggtaa

SEQ ID NO: 20 - DNA, 20 bp, synthetic construct
  source 1..20: mol_type = other DNA
caggactgggtgatggtgtc

SEQ ID NO: 21 - DNA, 20 bp, synthetic construct
  source 1..20: mol_type = other DNA
tctgagggtgagagcctgaa